European Patent Application EP 4 289 943 A1, published December 13, 2023. Title: Protein Deamidases. Applicant: Amano Enzyme Inc. The sequence listing filed with the application follows.

SEQUENCE LISTING (42 sequences)

SEQ ID NO: 1 - protein, 515 aa, Halobacteriovorax sp.
MSIFSIYSHATSVVFSDDLSFDNCKAPSKVPVVVCENGGKRAIVQINSRGHLLGLVTEGGTSKTFAVKQIVENGVPTYYNSLSDKINEERATSEFTTPITKLQEIAERKKSIEQAIEIAKKENSNILEDLEDFDSDLDDSLNKLKSVVAQASNLLWVNTKKDGNIHCEMSTKCPIKKCGDNHFFIFDPSRNIFMPINYTRDSRGNAKFTKSDSQITIARTMNGAVLELNDDYKTSRLTAARKAPQNLQSNPTAYFSFQDARFSDYLKTIIPHCSQNIKDDIISLGVQTNNERANLDFVHLVEVVNGTINSQYINKKFLPKNSCRDGDSYYTAESYKESQEFVPRSSGVISWKKAGELFEKAKKMKELTWRYTADGCYARAELMVNMMEEEGVIADKAWTSGYLKSKSSPHPWSYHVAPVVYVNNGRGHVQKMIIDPAVANGPVEPDEWLRLMGVNEKNLDQVGFPPSLDAVSVGRNTFTISDRSTFHPQDKTRLTKEQRVTAARALLADLGNRLQ

SEQ ID NO: 2 - protein, 564 aa, Halobacteriovoraceae bacterium
MNKLIKLPLFLIITLSSSFLWAEKVQVHIVDRDEPLECFHEESQYFCHDGENFLFGRNYGMDLYLTGSVDGSVDDFRVSSAVSLDNPDHILFEEREDPYRDSYEQVNRRPSYSKELMSLTMLENMTAPFSYDSESIALAKSNLYPLVQNRLDQIKNKFNQSNRIVKTEEGNELSCSQGSASAGQDVNCTFYQCTEEGSDKKYFYISDPNIQFGVHELFSVGTDGLPQREAIQSIHFPNDDKSILERFNFVPSAGQGFGEYTGQGDFLSSEYSYQKPQIDYEQMIPDFDNPKKSDAFKYLIGVNGRGAMENAVRGCSERTTRDFFYSIDDLMENVLARNSVQYITDFNNGLAGYYLSLENLPDIACSENGVFYNPSSYETARNVAAADRNSVQTISMEKARELFDKAQAMDDIAWGYKPDGCYARAHLMARRFEEMGITVDKAWLKGSLRAQGETPEEDIMWNFHVAPVVYVEHDNGEIERVVIDPSVEEGPVTAMEWAKNLSSDVEERVNITQFPYPENSAEYLKNSLAFSNSDPYLPLESTESTEEQKMSMAHATMLEYKGYE

SEQ ID NO: 3 - protein, 233 aa, Oryza sativa Japonica Group
MADDRVAVAGGATPPPPPPPPPLDASAFTHTPYYCEENVHLLCKELIRSGISDPAGTNLYAVFISNEEKKVPLWYQKASHSGDGFVLWDYHVICIQSRRKNGEVLDLVWDLDSSLPFPCSFIQYVSDAIRPLSFGNSTYRRLFRVIHAPVFLRSFASDRSHMKDHAGNWIQLPPKYESIVAEDGTTNNLNEYITMSMDDVKDLESMADDVYSSKHGVVINETILPEFFSRLPG

SEQ ID NO: 4 - protein, 309 aa, Acidobacteria bacterium
MPPTRESAVLTVANIREETGRILFHEREQIFSLPETDARAGISGRLREALERKTPVKAVLDPRRGIVQGITPAAEKEAGEFERSRTLLDKPGKTVSVNVAEIDPTRFNVVDLTLKSPIFKLCTKIVPSYTKAKEIFDFCAQQSCNLGIPTTVTPCIPFQYVRDDCYARAHKMRWIIEQRYGYCCEKVFSFANQNNDELSVRADKWGGCCVNWWYHVAPLIRVQIKISTFSFVIALVVDPSMFDKPVMLSSWLTAQENAACGAHAKVSMYSIQPGSAYTPANYAGTAFTTDPSYTATDATLIAYKNLTTC

SEQ ID NO: 5 - protein, 271 aa, Deltaproteobacteria bacterium
MSKSEVNSLFNDFLNHPKLVFSANNTGCESKADLMAEIAHQKGHEVSKIWVRPMNSTDNFPVYLNEAKTESTVWNYHVAIQVKMKTSSGTETMIIDPSLFDEPVTMDTWSKRISSLSDEYDYDLEFKESSREAFFGPEDMVTSETRARALAKRDDILSNSGNLNDPVVRDGYLMKLRGQYVDDLMKKNPQDFETLEELLLNQKFNMWFKTPLQIEQIKQLLDQKPRFYGIKSSDIKSKIDFSSPDASFELKKYFWKKIGKAFERLSSKSEE

SEQ ID NO: 6 - protein, 235 aa, Rhodospirillaceae bacterium
MAMTINPHLRDIFNLRRDRSGFFPVAEDAVRVVSPAQALEIFDTLRAMQNISHEYTDDGCAQRAHLMCRALVDMKLAPEKGWAFETPKRDLVVDYPHVSQIWWFHVAPVLRVASEKGGAEPMAFDTVLFDGPATMKEWGSVMKAQPEQIHVLPCGKSPKGHYGDYRPGVRTGYASDAAAQKAMDKYIALENEDGFVRPQVFESALRKKLEATTPDNPRPADRKKQPPAQGQNGPA

SEQ ID NO: 7 - protein, 303 aa, Flavobacterium alvei
MKKHPLLTSHKASILDLNTAKSLFAEITESGIPYDYQQANCHNISHYISSLLESKGYQCAKIWAFAPAVYSTSNSKLISFIDEKNISPTGTIDWRYHVAPVIEVQIGNKVRKMVIDLGLFPNEFVRYRTWLAKLKTKKLIYLIMDSEWYLYNSSMITNAQLEFDSNEEINANQPNIKLPEWFADKLITDFFKYEEESLEQHWVEKGLAVNETAIEFYDTEIKPILYSEQHQDLVKDYKMLVGDVFNFETIFRDNNWNYEMNNDFQIKHQEIISKYRTIYSLNLDKWKKALASLNEIILQKNIK

SEQ ID NO: 8 - protein, 380 aa, Embleya scabrispora
MKRERDLKNPSSQGVTAPTGERGPDDDTKRARTDAHTTDPAPAADSPAVQPAPDPTPAQPQPFRFTRAPGFLLAQQAEQKRAEAEEERRQGQLRAEQAGAEASTKPEPRTPAPMAEPKKDSSTLPDVRFAELSPKVIARMTPDQLSEAIEDRMENFGGLTPDTPLLTFRQTALVLGDDLPLAKSTMCVGQVHTWLHSRAALVPDVIPLCDAKASTLAAPATPAPTLAELTAVWRALTGSLVVPRSAAQDGCEFLAHAVCEWFENTHPDWARLHLCKRWVVAPSGGMHPPYHWKHHVAPQITCVEGPFVIDLLLGAQAPMACTAWVTAAKGASAPADTFEATAPWELLGAPASATAGFVPETLSPIGATLRTSIEACKRGW

SEQ ID NO: 9 - protein, 426 aa, Lentzea kentuckyensis
MPRENVLVDQVSELAIAAAAETRYHAVVFAGGSSARLDLEDSRATGWLAALEEMRAAGLSAYVEVDPGTGVIVELLCPLPVVVGELRESDDGVDVELVVSQARHRLSRGNPEFDELLAALRRARESQEPVLVTETLDAHEIIDVRSDPKVRTESVTTGESEVLGTPVTLAKANEMFTLVNNRTACSANPVAPGIPFTYPDDGCWGRAHEMCRLMIGAGVQPDKVWIYGSLHVVSFNKPGCNVYWGWHVAPTLTLTTGETYVVDPALFPNPVPRATWASVQGDPSASLVPTGADVFHRSSGGGLTFDPTYSQTNSVLATYRTQLQLRAAGPSGPPPYSECLTRPAGTQWFGTIAGNSSQRWFTFGWPAGWHMVWTIMPTLICPGTPTLSWSVAAERANSTQATYWITVTNSSPHTVRFEGRYDVLST

SEQ ID NO: 10 - protein, 350 aa, Streptomyces chilikensis
MRRSAREEIPAQGTDRALRRAPDRAEGAGARADSPPSAHPSALWALQRSAGNAAVTAVIQRMEGAAGKRKRSTSPEDQEAPKQARAATSSEEEYSSSSEEAETSSEEEREEPFSAQVMLQIANEQRRMTGLLEQMDERGAPDHIKRAAEDKLEILTLLRNLAPMRSVDTVHEAIRLLGMRPDSTAKTRYLAKLEEQLDYLAEEFPNAGPPTAETLRAMWPELVPAFGGAGGQVGEDGCEDRAHAICLAIARRSPAIAAHHLSKQWALPDGGLLHADHQWNHHVAASVTTANGVLVIDPVFSRSEPIELSRWAAMVQVDLDTNVHQVAWGFLGRPGADNLPDVNSAVEYVP

SEQ ID NO: 11 - protein, 591 aa, Streptomyces sp.
MADDGSAGTAISSTLLGRVARRKNISPLLLSNTSIEAGTRKRVELGLPKSEAEELTDRLAALLDAELLDEAGLQVWITDLCRLNPHAAEQFDETFEFRHRYAPVEAVIEAAGRGLLAEHLALELLGALHEAWQPPRVTDWLSAVALDGRPDPSPTPQIVALVAAVHEDLTRVGAGGSAKALRRIGALDRDLRALWALQRVWRQAYGTQLREELVSAFPGAEDQIAHLLAETTLDAVPAEVVDEWHQNLSRAHVLHPHQGPISLAYDYPDDGCQYRAHEATLLLHRWGAAVSKVVVVRRAGLSVTTENADGATPTRPGKVTWGWHIAPAVHRIKPDSTRQLVVLDPALSTEALPLDAWATAAGGSEKHANIYRGTLEQVREQILDDQERSFAEHTAVAVLPATVGSFEVGREAATLEDLDEQFRRWQITEILAAYSQQAADRRLARELDSFLRNPQHHGLAPEERSAALEQWLNGRSLHVATLRRYSRTAAALKEFTAPRTRLNALAVRALDRSDEAGWEDSDAELDTWESVAEIALHRGPVPGAGGEDFESLLSDHHQGGVRAFVDSDDEFEGEYDEGEDPSDLAAVPWGV

SEQ ID NO: 12 - DNA, 1548 bp, Halobacteriovorax sp.
atgagcatcttcagcatttacagccacgcgaccagcgtggttttcagcgacgatctgagctttgataactgcaaggcgccgagcaaagtgccggtggttgtgtgcgaaaacggtggcaagcgtgcgatcgtgcagattaacagccgtggtcacctgctgggcctggttaccgaaggtggcaccagcaagaccttcgcggttaaacaaattgtggagaacggtgttccgacctactataacagcctgagcgacaagatcaacgaggaacgtgcgaccagcgaatttaccaccccgatcaccaaactgcaggaaattgcggagcgtaagaaaagcattgaacaagcgatcgagattgcgaagaaagagaacagcaacatcctggaagatctggaggactttgatagcgacctggacgatagcctgaacaagctgaaaagcgttgtggcgcaggcgagcaacctgctgtgggttaacaccaagaaagacggtaacatccactgcgaaatgagcaccaaatgcccgattaagaaatgcggcgataaccacttctttatcttcgacccgagccgtaacatctttatgccgattaactacacccgtgatagccgtggtaacgcgaagttcaccaaaagcgacagccagatcaccattgcgcgtaccatgaacggcgcggtgctggagctgaacgacgattataagaccagccgtctgaccgcggcgcgtaaagcgccgcagaacctgcaaagcaacccgaccgcgtacttcagctttcaagatgcgcgttttagcgactatctgaagaccatcattccgcactgcagccagaacatcaaagacgatatcattagcctgggtgttcaaaccaacaacgaacgtgcgaacctggatttcgttcacctggttgaggtggtgaacggtaccatcaacagccagtacattaacaagaaatttctgccgaagaacagctgccgtgatggcgacagctactataccgcggagagctataaagaaagccaagagttcgtgccgcgtagcagcggtgttattagctggaagaaagcgggcgaactgtttgagaaggcgaagaaaatgaaagaactgacctggcgttacaccgcggatggttgctatgcgcgtgcggagctgatggtgaacatgatggaggaagagggtgttatcgcggacaaggcgtggaccagcggctacctgaagagcaaaagcagcccgcacccgtggagctaccatgtggcgccggttgtgtatgttaacaacggtcgtggccacgtgcagaagatgatcattgatccggcggtggcgaacggtccggttgaaccggacgagtggctgcgtctgatgggtgtgaacgagaagaacctggatcaagttggtttcccgccgagcctggatgcggttagcgtgggccgtaacaccttcaccatcagcgatcgtagcacctttcacccgcaggacaagacccgtctgaccaaagagcaacgtgttaccgcggcgcgtgcgctgctggcggacctgggtaaccgtctgcagtaa

SEQ ID NO: 13 - DNA, 1695 bp, Halobacteriovoraceae bacterium
atgaacaagctgatcaaactgccgctgttcctgatcattaccctgagcagcagctttctgtgggcggaaaaagtgcaggttcacattgtggaccgtgatgagccgctggaatgcttccacgaggaaagccaatacttttgccacgacggcgagaacttcctgtttggccgtaactacggtatggacctgtatctgaccggcagcgtggatggtagcgttgacgatttccgtgtgagcagcgcggttagcctggacaacccggatcacatcctgtttgaggaacgtgaggacccgtaccgtgatagctatgaacaggttaaccgtcgtccgagctacagcaaggagctgatgagcctgaccatgctggaaaacatgaccgcgccgttcagctacgacagcgaaagcattgcgctggcgaaaagcaacctgtatccgctggtgcagaaccgtctggatcaaatcaagaacaagttcaaccaaagcaaccgtattgttaagaccgaggaaggtaacgaactgagctgcagccagggcagcgcgagcgcgggtcaagacgtgaactgcaccttctaccagtgcaccgaggaaggcagcgacaagaaatacttttatatcagcgatccgaacattcaattcggtgtgcacgaactgtttagcgttggtaccgatggtctgccgcagcgtgaggcgatccaaagcattcacttcccgaacgacgataaaagcatcctggaacgtttcaactttgttccgagcgcgggtcagggcttcggcgagtacaccggccagggtgactttctgagcagcgaatacagctatcagaagccgcaaatcgattacgagcagatgattccggacttcgataacccgaagaaaagcgacgcgtttaaatatctgattggcgtgaacggccgtggtgcgatggagaacgcggttcgtggttgcagcgaacgtaccacccgtgatttcttttacagcatcgacgatctgatggaaaacgtgctggcgcgtaacagcgttcagtatattaccgacttcaacaacggcctggcgggttactatctgagcctggagaacctgccggatatcgcgtgcagcgaaaacggcgtgttttacaacccgagcagctatgaaaccgcgcgtaacgtggcggcggcggaccgtaacagcgttcagaccatcagcatggagaaggcgcgtgaactgttcgacaaagcgcaagcgatggacgatattgcgtggggctacaagccggatggttgctatgcgcgtgcgcacctgatggcgcgtcgttttgaggaaatgggtatcaccgttgacaaggcgtggctgaaaggcagcctgcgtgcgcagggtgaaaccccggaggaagatattatgtggaacttccacgtggcgccggtggtttacgttgagcacgacaacggcgagatcgaacgtgtggttattgatccgagcgtggaggaaggtccggttaccgcgatggagtgggcgaaaaacctgagcagcgacgtggaggaacgtgttaacatcacccagttcccgtacccggagaacagcgcggaatatctgaagaacagcctggcgtttagcaacagcgatccgtatctgccgctggagagcaccgaaagcaccgaggaacaaaagatgagcatggcgcacgcgaccatgctggagtacaaaggttatgaataa

SEQ ID NO: 14 - DNA, 702 bp, Oryza sativa Japonica Group
atggcggatgatcgtgttgcggttgcgggtggtgcgaccccgccgccgccgccgccgccgccgccgctggatgcgagcgcgtttacccacaccccgtactattgcgaggaaaacgtgcacctgctgtgcaaggagctgatccgtagcggtattagcgacccggcgggtaccaacctgtatgcggtgttcatcagcaacgaggaaaagaaagttccgctgtggtatcagaaggcgagccacagcggtgacggctttgtgctgtgggattaccacgttatctgcattcaaagccgtcgtaaaaacggtgaagtgctggacctggtttgggacctggatagcagcctgccgttcccgtgcagctttatccagtatgtgagcgatgcgattcgtccgctgagcttcggcaacagcacctaccgtcgtctgtttcgtgtgatccacgcgccggttttcctgcgtagctttgcgagcgaccgtagccacatgaaggatcacgcgggtaactggattcagctgccgccgaaatatgagagcattgttgcggaagacggcaccaccaacaacctgaacgagtacattaccatgagcatggacgatgtgaaggatctggaaagcatggcggacgatgtttatagcagcaaacacggtgttgttatcaatgagaccatcctgccggagttctttagccgcctgccgggttaa

SEQ ID NO: 15 - DNA, 930 bp, Acidobacteria bacterium
atgccgccaacccgtgagagcgcggttctgaccgtggcgaacatccgtgaggaaaccggtcgtattctgttccacgagcgtgaacagatctttagcctgccggaaaccgatgcgcgtgcgggtattagcggccgtctgcgtgaggcgctggagcgtaagaccccggttaaagcggtgctggacccgcgtcgtggtatcgtgcaaggcattaccccggcggcggagaaggaagcgggcgagttcgaacgtagccgtaccctgctggacaagccgggcaaaaccgtgagcgttaacgtggcggagatcgacccgacccgtttcaacgtggttgatctgaccctgaaaagcccgatctttaagctgtgcaccaaaattgttccgagctacaccaaggcgaaagaaatcttcgatttttgcgcgcagcaaagctgcaacctgggtatcccgaccaccgtgaccccgtgcattccgtttcagtacgttcgtgacgattgctatgcgcgtgcgcacaagatgcgttggatcattgagcagcgttacggctattgctgcgaaaaagtgttcagctttgcgaaccaaaacaacgacgagctgagcgttcgtgcggataagtggggtggctgctgcgttaactggtggtaccacgtggcgccgctgatccgtgttcaaatcaagattagcaccttcagctttgtgattgcgctggttgtggacccgagcatgttcgataaaccggttatgctgagcagctggctgaccgcgcaggaaaacgcggcgtgcggtgcgcacgcgaaagtgagcatgtatagcatccaaccgggtagcgcgtacaccccggcgaactatgcgggtaccgcgtttaccaccgacccgagctacaccgcgaccgatgcgaccctgattgcgtataaaaacctgaccacctgctaa

SEQ ID NO: 16 - DNA, 816 bp, Deltaproteobacteria bacterium
atgagcaagagcgaggtgaacagcctgttcaacgactttctgaaccacccgaagctggttttcagcgcgaacaacaccggttgcgaaagcaaagcggatctgatggcggagatcgcgcaccaaaagggccacgaagtgagcaaaatttgggttcgtccgatgaacagcaccgacaactttccggtgtacctgaacgaggcgaaaaccgaaagcaccgtttggaactatcacgtggcgatccaggttaagatgaaaaccagcagcggtaccgaaaccatgatcattgacccgagcctgttcgatgaaccggtgaccatggacacctggagcaagcgtattagcagcctgagcgatgaatacgactatgatctggagtttaaagaaagcagccgtgaggcgttctttggtccggaagacatggttaccagcgaaacccgtgcgcgtgcgctggcgaagcgtgacgatatcctgagcaacagcggcaacctgaacgacccggtggttcgtgatggttacctgatgaaactgcgtggccaatatgtggacgatctgatgaagaaaaacccgcaggatttcgaaaccctggaggaactgctgctgaaccaaaagttcaacatgtggtttaaaaccccgctgcagatcgaacaaattaagcagctgctggaccagaaaccgcgtttctacggtatcaagagcagcgatatcaagagcaaaattgactttagcagcccggatgcgagcttcgagctgaagaaatacttctggaagaaaattggcaaggcgtttgaacgtctgagcagcaaaagcgaggaataa

SEQ ID NO: 17 - DNA, 708 bp, Rhodospirillaceae bacterium
atggcgatgaccatcaacccgcacctgcgtgacattttcaacctgcgtcgtgatcgtagcggtttctttccggttgcggaggatgcggtgcgtgtggttagcccggcgcaggcgctggaaatctttgataccctgcgtgcgatgcaaaacattagccacgagtacaccgatgatggttgcgcgcagcgtgcgcacctgatgtgccgtgcgctggttgacatgaagctggcgccggagaaaggctgggcgttcgaaaccccgaagcgtgacctggtggttgattatccgcacgtgagccaaatctggtggtttcatgtggcgccggttctgcgtgtggcgagcgagaaaggtggcgcggaaccgatggcgttcgacaccgttctgtttgatggtccggcgaccatgaaggagtggggcagcgttatgaaagcgcagccggaacaaatccacgtgctgccgtgcggcaagagcccgaaaggtcactacggcgactatcgtccgggtgtgcgtaccggttatgcgagcgatgcggcggcgcagaaggcgatggataaatatattgcgctggagaacgaagatggcttcgttcgtccgcaagtgtttgagagcgcgctgcgtaagaaactggaagcgaccaccccggacaacccgcgtccggcggatcgtaagaaacagccgccggcgcagggtcaaaacggtccggcgtaa

SEQ ID NO: 18 - DNA, 912 bp, Flavobacterium alvei
atgaagaaacacccgctgctgaccagccacaaggcgagcatcctggatctgaacaccgcgaaaagcctgttcgcggaaatcaccgagagcggtattccgtacgactatcagcaagcgaactgccacaacatcagccactacattagcagcctgctggaaagcaagggctatcagtgcgcgaaaatttgggcgttcgcgccggcggtttacagcaccagcaacagcaagctgatcagctttattgatgagaaaaacatcagcccgaccggtaccattgactggcgttatcacgtggcgccggttatcgaagtgcaaattggtaacaaggttcgtaaaatggtgatcgatctgggcctgttcccgaacgagtttgtgcgttaccgtacctggctggcgaagctgaaaaccaagaaactgatctatctgattatggatagcgagtggtacctgtataacagcagcatgattaccaacgcgcagctggagttcgacagcaacgaggaaatcaacgcgaaccaaccgaacattaagctgccggaatggtttgcggacaagctgatcaccgatttctttaaatacgaggaagagagcctggaacagcactgggttgagaagggtctggcggtgaacgaaaccgcgattgagttttacgataccgaaatcaaaccgattctgtatagcgagcagcaccaagacctggttaaggattacaaaatgctggttggcgacgtgttcaactttgaaaccatcttccgtgataacaactggaactatgagatgaacaacgactttcagatcaagcaccaagaaatcatcagcaagtaccgtaccatctacagcctgaacctggacaaatggaagaaagcgctggcgagcctgaacgagatcattctgcaaaagaacatcaaataa

SEQ ID NO: 19 - DNA, 1143 bp, Embleya scabrispora
atgaagcgtgaacgtgatctgaaaaacccgagcagccagggtgtgaccgcgccgaccggcgagcgtggtccggacgatgacaccaagcgtgcgcgtaccgatgcgcacaccaccgacccggcgccggcggcggatagcccggcggttcaaccggcgccggacccgaccccggcgcagccgcaaccgttccgttttacccgtgcgccgggcttcctgctggcgcagcaagcggaacagaagcgtgcggaggcggaggaagagcgtcgtcagggtcaactgcgtgcggaacaggcgggtgcggaggcgagcaccaaaccggaaccgcgtaccccggcgccgatggcggagccgaagaaagatagcagcaccctgccggacgtgcgttttgcggaactgagcccgaaagttatcgcgcgtatgaccccggatcagctgagcgaagcgattgaggaccgtatggagaactttggtggcctgaccccggacaccccgctgctgacctttcgtcagaccgcgctggtgctgggtgatgacctgccgctggcgaagagcaccatgtgcgtgggccaagttcacacctggctgcacagccgtgcggcgctggtgccggatgttatcccgctgtgcgacgcgaaagcgagcaccctggcggcgccggcgaccccggcgccgaccctggcggagctgaccgcggtgtggcgtgcgctgaccggtagcctggtggttccgcgtagcgcggcgcaggatggttgcgagttcctggcgcacgcggtttgcgaatggtttgagaacacccacccggactgggcgcgtctgcacctgtgcaagcgttgggttgttgcgccgagcggtggcatgcacccgccgtaccactggaaacaccacgtggcgccgcagatcacctgcgtggaaggtccgttcgttattgatctgctgctgggtgcgcaagcgccgatggcgtgcaccgcgtgggttaccgcggcgaagggtgcgagcgcgccggcggacacctttgaagcgaccgcgccgtgggagctgctgggtgcgccggcgagcgcgaccgcgggctttgttccggaaaccctgagcccgatcggtgcgaccctgcgtaccagcattgaggcgtgcaaacgtggctggtaa

SEQ ID NO: 20 - DNA, 1281 bp, Lentzea kentuckyensis
atgccgcgtgagaacgttctggtggaccaggtgagcgagctggcgattgcggcggcggcggaaacccgttaccatgcggtggtttttgcgggtggcagcagcgcgcgtctggacctggaagatagccgtgcgaccggttggctggcggcgctggaggaaatgcgtgcggcgggtctgagcgcgtatgttgaggtggacccgggcaccggtgttattgtggaactgctgtgcccgctgccggtggttgtgggtgaactgcgtgaaagcgacgatggtgttgacgtggagctggttgtgagccaagcgcgtcaccgtctgagccgtggtaacccggagtttgatgaactgctggcggcgctgcgtcgtgcgcgtgagagccaagaaccggttctggtgaccgaaaccctggacgcgcacgaaatcattgacgttcgtagcgatccgaaggttcgtaccgagagcgtgaccaccggcgagagcgaagttctgggtaccccggtgaccctggcgaaagcgaacgaaatgttcaccctggtgaacaaccgtaccgcgtgcagcgcgaacccggttgcgccgggtatcccgtttacctatccggatgatggttgctggggtcgtgcgcacgagatgtgccgtctgatgatcggcgcgggtgttcagccggacaaagtgtggatttacggcagcctgcacgttgtgagcttcaacaaaccgggctgcaacgtttattggggttggcatgtggcgccgaccctgaccctgaccaccggtgaaacctatgttgtggacccggcgctgtttccgaacccggttccgcgtgcgacctgggcgagcgtgcagggcgacccgagcgcgagcctggttccgaccggtgcggatgtgttccaccgtagcagcggtggcggtctgacctttgacccgacctacagccaaaccaacagcgtgctggcgacctatcgtacccagctgcaactgcgtgcggcgggtccgagcggtccgccgccgtacagcgaatgcctgacccgtccggcgggtacccagtggttcggcaccatcgcgggtaacagcagccaacgttggttcacctttggttggccggcgggttggcacatggtgtggaccatcatgccgaccctgatttgcccgggtaccccgaccctgagctggagcgttgcggcggagcgtgcgaacagcacccaagcgacctactggattaccgttaccaacagcagcccgcacaccgtgcgttttgaaggtcgttatgatgttctgagcacctaa

SEQ ID NO: 21 - DNA, 1053 bp, Streptomyces chilikensis
atgcgtcgtagcgcgcgtgaggaaatcccggcgcagggtaccgaccgtgcgctgcgtcgtgcgccggatcgtgcggaaggcgcgggtgcgcgtgcggacagcccgccgagcgcgcacccgagcgcgctgtgggcgctgcaacgtagcgcgggtaacgcggcggtgaccgcggttattcaacgtatggagggtgcggcgggcaagcgtaaacgtagcaccagcccggaggatcaggaagcgccgaaacaggcgcgtgcggcgaccagcagcgaggaagagtacagcagcagcagcgaagaggcggaaaccagcagcgaagaggaacgtgaggaaccgttcagcgcgcaggtgatgctgcaaatcgcgaacgaacagcgtcgtatgaccggcctgctggagcaaatggacgaacgtggtgcgccggatcacatcaagcgtgcggcggaggacaaactggaaattctgaccctgctgcgtaacctggcgccgatgcgtagcgtggacaccgttcacgaggcgattcgtctgctgggcatgcgtccggatagcaccgcgaagacccgttacctggcgaaactggaggaacagctggattatctggcggaggagttcccgaacgcgggtccgccgaccgcggaaaccctgcgtgcgatgtggccggaactggtgccggcgtttggtggcgcgggtggccaagttggcgaggatggttgcgaagatcgtgcgcacgcgatctgcctggcgattgcgcgtcgtagcccggcgattgcggcgcaccacctgagcaagcagtgggcgctgccggatggtggcctgctgcacgcggatcaccaatggaaccatcatgtggcggcgagcgttaccaccgcgaacggtgtgctggttatcgacccggtgttcagccgtagcgagccgattgaactgagccgttgggcggcgatggtgcaggttgacctggataccaacgtgcaccaagttgcgtggggttttctgggccgtccgggtgcggacaacctgccggatgttaacagcgcggtggaatatgttccgtaa

SEQ ID NO: 22 - DNA, 1776 bp, Streptomyces sp.
atggcggatgatggtagcgcgggtaccgcgatcagcagcaccctgctgggtcgtgttgcgcgtcgtaagaacatcagcccgctgctgctgagcaacaccagcattgaagcgggtacccgtaagcgtgtggaactgggcctgccgaaaagcgaagcggaggaactgaccgaccgtctggcggcgctgctggatgcggaactgctggatgaggcgggcctgcaagtttggatcaccgacctgtgccgtctgaacccgcacgcggcggagcagtttgatgaaaccttcgagtttcgtcaccgttacgcgccggtggaagcggttattgaggcggcgggtcgtggcctgctggcggaacatctggcgctggagctgctgggtgcgctgcatgaagcgtggcaaccgccgcgtgttaccgactggctgagcgcggtggcgctggatggtcgtccggacccgagcccgaccccgcagattgtggcgctggttgcggcggtgcatgaggatctgacccgtgttggtgcgggtggcagcgcgaaagcgctgcgtcgtattggtgcgctggaccgtgatctgcgtgcgctgtgggcgctgcagcgtgtttggcgtcaagcgtacggtacccagctgcgtgaagaactggtgagcgcgttcccgggtgcggaagaccaaatcgcgcacctgctggcggaaaccaccctggatgcggttccggcggaagtggttgatgagtggcaccaaaacctgagccgtgcgcatgtgctgcacccgcaccagggtccgattagcctggcgtacgactatccggacgatggctgccagtatcgtgcgcacgaagcgaccctgctgctgcaccgttggggtgcggcggttagcaaggtggttgtggttcgtcgtgcgggtctgagcgtgaccaccgagaacgcggatggtgcgaccccgacccgtccgggcaaggttacctggggctggcacattgcgccggcggtgcaccgtattaaaccggacagcacccgtcaactggtggttctggacccggcgctgagcaccgaagcgctgccgctggatgcgtgggcgaccgcggcgggtggcagcgagaaacacgcgaacatctaccgtggtaccctggaacaggttcgtgagcaaattctggacgatcaggaacgtagctttgcggagcacaccgcggtggcggttctgccggcgaccgttggtagctttgaagttggtcgtgaggcggcgaccctggaagacctggatgagcaattccgtcgttggcagatcaccgaaattctggcggcgtacagccaacaagcggcggaccgtcgtctggcgcgtgagctggatagctttctgcgtaacccgcaacaccatggtctggcgccggaggaacgtagcgcggcgctggaacagtggctgaacggccgtagcctgcatgttgcgaccctgcgtcgttatagccgtaccgcggcggcgctgaaggagttcaccgcgccgcgtacccgtctgaacgcgctggcggtgcgtgcgctggaccgtagcgatgaagcgggttgggaggacagcgatgcggagctggacacctgggaaagcgttgcggagattgcgctgcaccgtggtccggtgccgggtgcgggtggcgaagactttgagagcctgctgagcgatcaccaccagggtggcgttcgtgcgttcgtggacagcgacgatgagtttgaaggcgagtatgatgagggtgaggacccgagcgatctggcggcggttccgtggggcgtgtaa

SEQ ID NO: 23 - protein, 179 aa, Halobacteriovorax sp.
MSQEFVPRSSGVISWKKAGELFEKAKKMKELTWRYTADGCYARAELMVNMMEEEGVIADKAWTSGYLKSKSSPHPWSYHVAPVVYVNNGRGHVQKMIIDPAVANGPVEPDEWLRLMGVNEKNLDQVGFPPSLDAVSVGRNTFTISDRSTFHPQDKTRLTKEQRVTAARALLADLGNRLQ

SEQ ID NO: 24 - protein, 185 aa, Halobacteriovoraceae bacterium
MRNVAAADRNSVQTISMEKARELFDKAQAMDDIAWGYKPDGCYARAHLMARRFEEMGITVDKAWLKGSLRAQGETPEEDIMWNFHVAPVVYVEHDNGEIERVVIDPSVEEGPVTAMEWAKNLSSDVEERVNITQFPYPENSAEYLKNSLAFSNSDPYLPLESTESTEEQKMSMAHATMLEYKGYE

SEQ ID NO: 25 - protein, 189 aa, Acidobacteria bacterium
MCTKIVPSYTKAKEIFDFCAQQSCNLGIPTTVTPCIPFQYVRDDCYARAHKMRWIIEQRYGYCCEKVFSFANQNNDELSVRADKWGGCCVNWWYHVAPLIRVQIKISTFSFVIALVVDPSMFDKPVMLSSWLTAQENAACGAHAKVSMYSIQPGSAYTPANYAGTAFTTDPSYTATDATLIAYKNLTTC

SEQ ID NO: 26 - protein, 146 aa, Deltaproteobacteria bacterium
MSKSEVNSLFNDFLNHPKLVFSANNTGCESKADLMAEIAHQKGHEVSKIWVRPMNSTDNFPVYLNEAKTESTVWNYHVAIQVKMKTSSGTETMIIDPSLFDEPVTMDTWSKRISSLSDEYDYDLEFKESSREAFFGPEDMVTSETR

SEQ ID NO: 27 - protein, 218 aa, Rhodospirillaceae bacterium
MRSGFFPVAEDAVRVVSPAQALEIFDTLRAMQNISHEYTDDGCAQRAHLMCRALVDMKLAPEKGWAFETPKRDLVVDYPHVSQIWWFHVAPVLRVASEKGGAEPMAFDTVLFDGPATMKEWGSVMKAQPEQIHVLPCGKSPKGHYGDYRPGVRTGYASDAAAQKAMDKYIALENEDGFVRPQVFESALRKKLEATTPDNPRPADRKKQPPAQGQNGPA

SEQ ID NO: 28 - protein, 188 aa, Rhodospirillaceae bacterium
MRSGFFPVAEDAVRVVSPAQALEIFDTLRAMQNISHEYTDDGCAQRAHLMCRALVDMKLAPEKGWAFETPKRDLVVDYPHVSQIWWFHVAPVLRVASEKGGAEPMAFDTVLFDGPATMKEWGSVMKAQPEQIHVLPCGKSPKGHYGDYRPGVRTGYASDAAAQKAMDKYIALENEDGFVRPQVFESAL

SEQ ID NO: 29 - protein, 295 aa, Flavobacterium alvei
MHKASILDLNTAKSLFAEITESGIPYDYQQANCHNISHYISSLLESKGYQCAKIWAFAPAVYSTSNSKLISFIDEKNISPTGTIDWRYHVAPVIEVQIGNKVRKMVIDLGLFPNEFVRYRTWLAKLKTKKLIYLIMDSEWYLYNSSMITNAQLEFDSNEEINANQPNIKLPEWFADKLITDFFKYEEESLEQHWVEKGLAVNETAIEFYDTEIKPILYSEQHQDLVKDYKMLVGDVFNFETIFRDNNWNYEMNNDFQIKHQEIISKYRTIYSLNLDKWKKALASLNEIILQKNIK

SEQ ID NO: 30 - protein, 178 aa, Flavobacterium alvei
MHKASILDLNTAKSLFAEITESGIPYDYQQANCHNISHYISSLLESKGYQCAKIWAFAPAVYSTSNSKLISFIDEKNISPTGTIDWRYHVAPVIEVQIGNKVRKMVIDLGLFPNEFVRYRTWLAKLKTKKLIYLIMDSEWYLYNSSMITNAQLEFDSNEEINANQPNIKLPEWFADKL

SEQ ID NO: 31 - protein, 266 aa, Lentzea kentuckyensis
MVLGTPVTLAKANEMFTLVNNRTACSANPVAPGIPFTYPDDGCWGRAHEMCRLMIGAGVQPDKVWIYGSLHVVSFNKPGCNVYWGWHVAPTLTLTTGETYVVDPALFPNPVPRATWASVQGDPSASLVPTGADVFHRSSGGGLTFDPTYSQTNSVLATYRTQLQLRAAGPSGPPPYSECLTRPAGTQWFGTIAGNSSQRWFTFGWPAGWHMVWTIMPTLICPGTPTLSWSVAAERANSTQATYWITVTNSSPHTVRFEGRYDVLST

SEQ ID NO: 32 - protein, 181 aa, Lentzea kentuckyensis
MVLGTPVTLAKANEMFTLVNNRTACSANPVAPGIPFTYPDDGCWGRAHEMCRLMIGAGVQPDKVWIYGSLHVVSFNKPGCNVYWGWHVAPTLTLTTGETYVVDPALFPNPVPRATWASVQGDPSASLVPTGADVFHRSSGGGLTFDPTYSQTNSVLATYRTQLQLRAAGPSGPPPYSECLT

SEQ ID NO: 33 - DNA, 540 bp, Halobacteriovorax sp.
atgagccaagagttcgtgccgcgtagcagcggtgttattagctggaagaaagcgggcgaactgtttgagaaggcgaagaaaatgaaagaactgacctggcgttacaccgcggatggttgctatgcgcgtgcggagctgatggtgaacatgatggaggaagagggtgttatcgcggacaaggcgtggaccagcggctacctgaagagcaaaagcagcccgcacccgtggagctaccatgtggcgccggttgtgtatgttaacaacggtcgtggccacgtgcagaagatgatcattgatccggcggtggcgaacggtccggttgaaccggacgagtggctgcgtctgatgggtgtgaacgagaagaacctggatcaagttggtttcccgccgagcctggatgcggttagcgtgggccgtaacaccttcaccatcagcgatcgtagcacctttcacccgcaggacaagacccgtctgaccaaagagcaacgtgttaccgcggcgcgtgcgctgctggcggacctgggtaaccgtctgcagtaa

SEQ ID NO: 34 - DNA, 558 bp, Halobacteriovoraceae bacterium
atgcgtaacgtggcggcggcggaccgtaacagcgttcagaccatcagcatggagaaggcgcgtgaactgttcgacaaagcgcaagcgatggacgatattgcgtggggctacaagccggatggttgctatgcgcgtgcgcacctgatggcgcgtcgttttgaggaaatgggtatcaccgttgacaaggcgtggctgaaaggcagcctgcgtgcgcagggtgaaaccccggaggaagatattatgtggaacttccacgtggcgccggtggtttacgttgagcacgacaacggcgagatcgaacgtgtggttattgatccgagcgtggaggaaggtccggttaccgcgatggagtgggcgaaaaacctgagcagcgacgtggaggaacgtgttaacatcacccagttcccgtacccggagaacagcgcggaatatctgaagaacagcctggcgtttagcaacagcgatccgtatctgccgctggagagcaccgaaagcaccgaggaacaaaagatgagcatggcgcacgcgaccatgctggagtacaaaggttatgaataa

SEQ ID NO: 35 - DNA, 570 bp, Acidobacteria bacterium
atgtgcaccaaaattgttccgagctacaccaaggcgaaagaaatcttcgatttttgcgcgcagcaaagctgcaacctgggtatcccgaccaccgtgaccccgtgcattccgtttcagtacgttcgtgacgattgctatgcgcgtgcgcacaagatgcgttggatcattgagcagcgttacggctattgctgcgaaaaagtgttcagctttgcgaaccaaaacaacgacgagctgagcgttcgtgcggataagtggggtggctgctgcgttaactggtggtaccacgtggcgccgctgatccgtgttcaaatcaagattagcaccttcagctttgtgattgcgctggttgtggacccgagcatgttcgataaaccggttatgctgagcagctggctgaccgcgcaggaaaacgcggcgtgcggtgcgcacgcgaaagtgagcatgtatagcatccaaccgggtagcgcgtacaccccggcgaactatgcgggtaccgcgtttaccaccgacccgagctacaccgcgaccgatgcgaccctgattgcgtataaaaacctgaccacctgctaa

SEQ ID NO: 36 - DNA, 441 bp, Deltaproteobacteria bacterium
atgagcaagagcgaggtgaacagcctgttcaacgactttctgaaccacccgaagctggttttcagcgcgaacaacaccggttgcgaaagcaaagcggatctgatggcggagatcgcgcaccaaaagggccacgaagtgagcaaaatttgggttcgtccgatgaacagcaccgacaactttccggtgtacctgaacgaggcgaaaaccgaaagcaccgtttggaactatcacgtggcgatccaggttaagatgaaaaccagcagcggtaccgaaaccatgatcattgacccgagcctgttcgatgaaccggtgaccatggacacctggagcaagcgtattagcagcctgagcgatgaatacgactatgatctggagtttaaagaaagcagccgtgaggcgttctttggtccggaagacatggttaccagcgaaacccgttag

SEQ ID NO: 37 - DNA, 657 bp, Rhodospirillaceae bacterium
atgcgtagcggtttctttccggttgcggaggatgcggtgcgtgtggttagcccggcgcaggcgctggaaatctttgataccctgcgtgcgatgcaaaacattagccacgagtacaccgatgatggttgcgcgcagcgtgcgcacctgatgtgccgtgcgctggttgacatgaagctggcgccggagaaaggctgggcgttcgaaaccccgaagcgtgacctggtggttgattatccgcacgtgagccaaatctggtggtttcatgtggcgccggttctgcgtgtggcgagcgagaaaggtggcgcggaaccgatggcgttcgacaccgttctgtttgatggtccggcgaccatgaaggagtggggcagcgttatgaaagcgcagccggaacaaatccacgtgctgccgtgcggcaagagcccgaaaggtcactacggcgactatcgtccgggtgtgcgtaccggttatgcgagcgatgcggcggcgcagaaggcgatggataaatatattgcgctggagaacgaagatggcttcgttcgtccgcaagtgtttgagagcgcgctgcgtaagaaactggaagcgaccaccccggacaacccgcgtccggcggatcgtaagaaacagccgccggcgcagggtcaaaacggtccggcgtaa

SEQ ID NO: 38 - DNA, 567 bp, Rhodospirillaceae bacterium
atgcgtagcggtttctttccggttgcggaggatgcggtgcgtgtggttagcccggcgcaggcgctggaaatctttgataccctgcgtgcgatgcaaaacattagccacgagtacaccgatgatggttgcgcgcagcgtgcgcacctgatgtgccgtgcgctggttgacatgaagctggcgccggagaaaggctgggcgttcgaaaccccgaagcgtgacctggtggttgattatccgcacgtgagccaaatctggtggtttcatgtggcgccggttctgcgtgtggcgagcgagaaaggtggcgcggaaccgatggcgttcgacaccgttctgtttgatggtccggcgaccatgaaggagtggggcagcgttatgaaagcgcagccggaacaaatccacgtgctgccgtgcggcaagagcccgaaaggtcactacggcgactatcgtccgggtgtgcgtaccggttatgcgagcgatgcggcggcgcagaaggcgatggataaatatattgcgctggagaacgaagatggcttcgttcgtccgcaagtgtttgagagcgcgctgtag

SEQ ID NO: 39 - DNA, 888 bp, Flavobacterium alvei
atgcacaaggcgagcatcctggatctgaacaccgcgaaaagcctgttcgcggaaatcaccgagagcggtattccgtacgactatcagcaagcgaactgccacaacatcagccactacattagcagcctgctggaaagcaagggctatcagtgcgcgaaaatttgggcgttcgcgccggcggtttacagcaccagcaacagcaagctgatcagctttattgatgagaaaaacatcagcccgaccggtaccattgactggcgttatcacgtggcgccggttatcgaagtgcaaattggtaacaaggttcgtaaaatggtgatcgatctgggcctgttcccgaacgagtttgtgcgttaccgtacctggctggcgaagctgaaaaccaagaaactgatctatctgattatggatagcgagtggtacctgtataacagcagcatgattaccaacgcgcagctggagttcgacagcaacgaggaaatcaacgcgaaccaaccgaacattaagctgccggaatggtttgcggacaagctgatcaccgatttctttaaatacgaggaagagagcctggaacagcactgggttgagaagggtctggcggtgaacgaaaccgcgattgagttttacgataccgaaatcaaaccgattctgtatagcgagcagcaccaagacctggttaaggattacaaaatgctggttggcgacgtgttcaactttgaaaccatcttccgtgataacaactggaactatgagatgaacaacgactttcagatcaagcaccaagaaatcatcagcaagtaccgtaccatctacagcctgaacctggacaaatggaagaaagcgctggcgagcctgaacgagatcattctgcaaaagaacatcaaataa

SEQ ID NO: 40 - DNA, 537 bp, Flavobacterium alvei
atgcacaaggcgagcatcctggatctgaacaccgcgaaaagcctgttcgcggaaatcaccgagagcggtattccgtacgactatcagcaagcgaactgccacaacatcagccactacattagcagcctgctggaaagcaagggctatcagtgcgcgaaaatttgggcgttcgcgccggcggtttacagcaccagcaacagcaagctgatcagctttattgatgagaaaaacatcagcccgaccggtaccattgactggcgttatcacgtggcgccggttatcgaagtgcaaattggtaacaaggttcgtaaaatggtgatcgatctgggcctgttcccgaacgagtttgtgcgttaccgtacctggctggcgaagctgaaaaccaagaaactgatctatctgattatggatagcgagtggtacctgtataacagcagcatgattaccaacgcgcagctggagttcgacagcaacgaggaaatcaacgcgaaccaaccgaacattaagctgccggaatggtttgcggacaagctgtag

SEQ ID NO: 41 - DNA, 801 bp, Lentzea kentuckyensis
atggttctgggtaccccggtgaccctggcgaaagcgaacgaaatgttcaccctggtgaacaaccgtaccgcgtgcagcgcgaacccggttgcgccgggtatcccgtttacctatccggatgatggttgctggggtcgtgcgcacgagatgtgccgtctgatgatcggcgcgggtgttcagccggacaaagtgtggatttacggcagcctgcacgttgtgagcttcaacaaaccgggctgcaacgtttattggggttggcatgtggcgccgaccctgaccctgaccaccggtgaaacctatgttgtggacccggcgctgtttccgaacccggttccgcgtgcgacctgggcgagcgtgcagggcgacccgagcgcgagcctggttccgaccggtgcggatgtgttccaccgtagcagcggtggcggtctgacctttgacccgacctacagccaaaccaacagcgtgctggcgacctatcgtacccagctgcaactgcgtgcggcgggtccgagcggtccgccgccgtacagcgaatgcctgacccgtccggcgggtacccagtggttcggcaccatcgcgggtaacagcagccaacgttggttcacctttggttggccggcgggttggcacatggtgtggaccatcatgccgaccctgatttgcccgggtaccccgaccctgagctggagcgttgcggcggagcgtgcgaacagcacccaagcgacctactggattaccgttaccaacagcagcccgcacaccgtgcgttttgaaggtcgttatgatgttctgagcacctaa

SEQ ID NO: 42 - DNA, 546 bp, Lentzea kentuckyensis
atggttctgggtaccccggtgaccctggcgaaagcgaacgaaatgttcaccctggtgaacaaccgtaccgcgtgcagcgcgaacccggttgcgccgggtatcccgtttacctatccggatgatggttgctggggtcgtgcgcacgagatgtgccgtctgatgatcggcgcgggtgttcagccggacaaagtgtggatttacggcagcctgcacgttgtgagcttcaacaaaccgggctgcaacgtttattggggttggcatgtggcgccgaccctgaccctgaccaccggtgaaacctatgttgtggacccggcgctgtttccgaacccggttccgcgtgcgacctgggcgagcgtgcagggcgacccgagcgcgagcctggttccgaccggtgcggatgtgttccaccgtagcagcggtggcggtctgacctttgacccgacctacagccaaaccaacagcgtgctggcgacctatcgtacccagctgcaactgcgtgcggcgggtccgagcggtccgccgccgtacagcgaatgcctgacctag